European Patent Application EP 4 785 953 A1, published August 5, 2026. Title: 一种双特异性抗体在制备治疗癌症的药物中的用途. Applicant: 上海翰森生物医药科技有限公司. The sequence listing filed with the application follows.

SEQUENCE LISTING (24 sequences)

SEQ ID NO: 1 - protein, 10 aa, synthetic construct
GGSVTSVNYY

SEQ ID NO: 2 - protein, 7 aa, synthetic construct
ISYSGNT

SEQ ID NO: 3 - protein, 10 aa, synthetic construct
VRAPYYYMDV

SEQ ID NO: 4 - protein, 6 aa, synthetic construct
QGISSW

SEQ ID NO: 5 - skipped

SEQ ID NO: 6 - protein, 9 aa, synthetic construct
QQANSFPLT

SEQ ID NO: 7 - protein, 118 aa, synthetic construct
EVQLQESGPGLVKPSETLSLTCTVSGGSVTSVNYYWKWIRQPPGKGLEWIGYISYSGNTNYNPSLKSRVTISVDTSKNQFSLKLSSVTAADTAVYYCVRAPYYYMDVWSKGTTVTVSS

SEQ ID NO: 8 - protein, 107 aa, synthetic construct
DIVMTQSPSSVSASVGDRVTITCRASQGISSWLAWYQQKPGKAPKLLIYAVSSLQSGVPSRFSGSGSGTDFTLTISSLQPEDFATYFCQQANSFPLTFGGGTKVEIK

SEQ ID NO: 9 - protein, 8 aa, synthetic construct
GFTFSTYG

SEQ ID NO: 10 - protein, 8 aa, synthetic construct
IWDDGSYK

SEQ ID NO: 11 - protein, 18 aa, synthetic construct
ARDGITMVRGVMKDYFDY

SEQ ID NO: 12 - protein, 6 aa, synthetic construct
QDISSA

SEQ ID NO: 13 - skipped

SEQ ID NO: 14 - protein, 9 aa, synthetic construct
QQFNSYPLT

SEQ ID NO: 15 - protein, 125 aa, synthetic construct
EVQLVESGGGVVQPGRSLRLSCAASGFTFSTYGMHWVRQAPGKGLEWVAVIWDDGSYKYYGDSVKGRFTISRDNSKNTLYLQMNSLRAEDTAVYYCARDGITMVRGVMKDYFDYWGQGTLVTVSS

SEQ ID NO: 16 - protein, 107 aa, synthetic construct
DIQLTQSPSSLSASVGDRVTITCRASQDISSALVWYQQKPGKAPKLLIYDASSLESGVPSRFSGSESGTDFTLTISSLQPEDFATYYCQQFNSYPLTFGGGTKVEIK

SEQ ID NO: 17 - protein, 329 aa, synthetic construct
ASTKGPSVFPLAPSSKSTSGGTAALGCQVEDYFPEPVTVSWNSGALTSGVHTFPAVLQSSGLYELSSVVTVPSSSLGTQTYICNVNHKPSNTKVDKKVEPKSCDKTHTCPPCPAPELLGGPSVFLFPPKPKDTLMISRTPEVTCVVVDVSHEDPEVKFNWYVDGVEVHNAKTKPREEQYNSTYRVVSVLTVLHQDWLNGKEYKCKVSNKALPAPIEKTISKAKGQPREPQVYTLPPCRDELTKNQVSLWCLVKGFYPSDIAVEWESNGQPENNYKTTPPVLDSDGSFFLYSKLTVDKSRWQQGNVFSCSVMHEALHNHYTQKSLSLSPG

SEQ ID NO: 18 - protein, 329 aa, synthetic construct
ASTKGPSVFPRAPSSKSTSGGTAALGCLVRDYFPEPVTVSWNSGALTSGVHTFPAVLQSSGLYSLSSVVTVPSSSLGTQTYICNVNHKPSNTKVDKKVEPKSCDKTHTCPPCPAPELLGGPSVFLFPPKPKDTLMISRTPEVTCVVVDVSHEDPEVKFNWYVDGVEVHNAKTKPREEQYNSTYRVVSVLTVLHQDWLNGKEYKCKVSNKALPAPIEKTISKAKGQPREPQVCTLPPSRDELTKNQVSLSCAVKGFYPSDIAVEWESNGQPENNYKTTPPVLDSDGSFFLVSKLTVDKSRWQQGNVFSCSVMHEALHNHYTQKSLSLSPG

SEQ ID NO: 19 - protein, 107 aa, synthetic construct
RTVAAPSVFIFPPSDEQLKSGRASVVCLLNNFYPREAKVQWKVDNALQSGNSQESVTEQDSKDSTYSLSSRLQLSKADYEKHKVYACEVTHQGLSSPVTKSFNRGEC

SEQ ID NO: 20 - protein, 107 aa, synthetic construct
RTVAAPSVFIFPPSDEELKSGTASVQCLLNNFYPREAKVQWKVDNALQSGNSQESVTEQDSKDSTYSLSSELTLSKADYEKHKVYACEVTHQGLSSPVTKSFNRGEC

SEQ ID NO: 21 - protein, 447 aa, synthetic construct
EVQLQESGPGLVKPSETLSLTCTVSGGSVTSVNYYWKWIRQPPGKGLEWIGYISYSGNTNYNPSLKSRVTISVDTSKNQFSLKLSSVTAADTAVYYCVRAPYYYMDVWSKGTTVTVSSASTKGPSVFPLAPSSKSTSGGTAALGCQVEDYFPEPVTVSWNSGALTSGVHTFPAVLQSSGLYELSSVVTVPSSSLGTQTYICNVNHKPSNTKVDKKVEPKSCDKTHTCPPCPAPELLGGPSVFLFPPKPKDTLMISRTPEVTCVVVDVSHEDPEVKFNWYVDGVEVHNAKTKPREEQYNSTYRVVSVLTVLHQDWLNGKEYKCKVSNKALPAPIEKTISKAKGQPREPQVYTLPPCRDELTKNQVSLWCLVKGFYPSDIAVEWESNGQPENNYKTTPPVLDSDGSFFLYSKLTVDKSRWQQGNVFSCSVMHEALHNHYTQKSLSLSPG

SEQ ID NO: 22 - protein, 214 aa, synthetic construct
DIVMTQSPSSVSASVGDRVTITCRASQGISSWLAWYQQKPGKAPKLLIYAVSSLQSGVPSRFSGSGSGTDFTLTISSLQPEDFATYFCQQANSFPLTFGGGTKVEIKRTVAAPSVFIFPPSDEQLKSGRASVVCLLNNFYPREAKVQWKVDNALQSGNSQESVTEQDSKDSTYSLSSRLQLSKADYEKHKVYACEVTHQGLSSPVTKSFNRGEC

SEQ ID NO: 23 - protein, 454 aa, synthetic construct
EVQLVESGGGVVQPGRSLRLSCAASGFTFSTYGMHWVRQAPGKGLEWVAVIWDDGSYKYYGDSVKGRFTISRDNSKNTLYLQMNSLRAEDTAVYYCARDGITMVRGVMKDYFDYWGQGTLVTVSSASTKGPSVFPRAPSSKSTSGGTAALGCLVRDYFPEPVTVSWNSGALTSGVHTFPAVLQSSGLYSLSSVVTVPSSSLGTQTYICNVNHKPSNTKVDKKVEPKSCDKTHTCPPCPAPELLGGPSVFLFPPKPKDTLMISRTPEVTCVVVDVSHEDPEVKFNWYVDGVEVHNAKTKPREEQYNSTYRVVSVLTVLHQDWLNGKEYKCKVSNKALPAPIEKTISKAKGQPREPQVCTLPPSRDELTKNQVSLSCAVKGFYPSDIAVEWESNGQPENNYKTTPPVLDSDGSFFLVSKLTVDKSRWQQGNVFSCSVMHEALHNHYTQKSLSLSPG

SEQ ID NO: 24 - protein, 214 aa, synthetic construct
DIQLTQSPSSLSASVGDRVTITCRASQDISSALVWYQQKPGKAPKLLIYDASSLESGVPSRFSGSESGTDFTLTISSLQPEDFATYYCQQFNSYPLTFGGGTKVEIKRTVAAPSVFIFPPSDEELKSGTASVQCLLNNFYPREAKVQWKVDNALQSGNSQESVTEQDSKDSTYSLSSELTLSKADYEKHKVYACEVTHQGLSSPVTKSFNRGEC